European Patent Specification EP 4 055 177 B1, published July 31, 2024. Title: FILAMENTOUS FUNGAL STRAINS COMPRISING ENHANCED PROTEIN PRODUCITIVTY PHENOTYPES AND METHODS THEREOF. Applicant: DANISCO US INC. The sequence listing filed with the application follows.

SEQUENCE LISTING (19 sequences)

SEQ ID NO: 1 - DNA, 6143 bp, Hypocrea jecorina
atggacccggacccggacctgcacctgccagcacgagtagagcgcgcgagcctggatggtagcgtgtttgtagcccacgatgcgcatccgccggctcgccatctgccccatctccatctcccccagctggcccatccagcctcaaactcaacctccaacttcaccttgcgctcgcactcgcactcgcccgctgccggcgacgtcgtcctgcccgcctcaaccgccaatgcccacgtcctcgcccaccatgcagctgccaccctagatcctgacgactactacaggagctacgagacagcctccagccccggcggcgagccacaatcgctcccaatggcctcgccagtcccgcctcccacgccggatggggctgctgcaagacacctgcagccgcctgcaaatcgcagtgctggccgtcagggtaccagtaataccgccgtgcgctccgcctcgagccccctcgaccgcaggccagccgcggcggcgccgtcgtcaagatccccctcggccagcgcccccagcgtgagggatctgaagaagcgcttcgatcagaacagcggccccaactccatcccaagagctcctccacgccaggctgcaccggtggcccgggtcagcaagcaagagtccagcaaacccaagcccaagcccaagcccagcctgtcggccccttcgtccacgcacccaggctctcgctcggcggtccccgcttccaactcgtccaagcaatctcggtcgtcgtcgtcgtccaactcagcctcgacctcgcgctcgacgtcgacgccggccccgtcagcccgctcgcagaagccacggcacgttgagcgcgagcaggcggcgggaagttcgcggtcgtttgcaaaccgtattgggaaccatcagcctgagacatccactactaacgggaactcgaacgcctccagctctatgacaccacgcccacacaagtccccaccctcagcctcccagccgtcgccgccatccccaaagtctaatcctcagttcccgggcctcctgtttggcgaaatccccccgggccagctcgacgttgccgcgccaggctttggcatcgacaacatccgcccgcgacgaacgtccgaatccaacgtgcacggcctcgcggggcgtcaacgcagcctctccgacctcgaagccgagcccgcgtccccgtccagctggtacagggacgtccacatgtcccgagggagcacgccgaaaacccacgcgcgatctcgcagcgatctctcggcgctgaagcccatcctcacaaccttgcatcccaagtcgcctacgcccgcatcggcgtcggcatcagcaaagacaagggcgaaatcaccaacagtagctgctttcgcggcagccacggtaacggcaacggctgtcgcagcaggggccgcggccgccaccccttcggtctcgcacgcgtcggcagccgccagctccaaactccccgtttccatcagcaggaggcttgcgagcccaaccaactccagtcctacctcttcgcgatcagcctcgccctctgcgcttcgcagactgccagccaatggtcgtagcaatagcagacaggccaaaccgatcgcccccacgaaccgagcgaaaacacccacgcagacgggtcgaaagcagcctccccaggggctcgttacaccgagtaatagcaacaaccggctccaagcgtacgtgtccaccgcaccacccaagctctcaccgccattgaggagctctcgaccgcgacagccagtctccgtagcgacgacagcaagctcccggatgaaagaggcggcggccaaggcgaagccccctgcacggccaaatgcacgggacggcccttcgtcgtccaagacgtacgatccggcgaagcgtaaaatcatagtgggacccatagacttcgagcagcgtcgggaacacattcgactggcatacaccaagaccattcgcgaaagccaggcctttgaggtgcgccagaaagcggtggagaggaggcggaagcagatggaggaggccaaatcggaagccgcagccaccgaagctacagcgacaagtagcacagctacaggcccatctacgtctgcggattcaccgaccacggtgactgctggagatgacgaggcgacgaataaggggccctcggacggccatgcacgagtaattccagaagtaatagcggcagagacagggctggtcgcgagcccctcggcacaggagccggctgtggaactcccagctgatcatggctctcgcgctgctgtggagaaccagggaacccttctagaaatcccgacagatgcagcctcgcacccggcatctggcaagggtgatgattcgccgacgctgggcatccccgggggcttcccagaaccctcaccgtcctccgccgcggccagaacgcagcggcctctgtcgaccatttcaatcatttcagccacgtctgctgttacggagtttgatacagagccccaggcggagctcgccgacctggctatgtccgatcggccgctcagcccccagatcatagtgccgacgagggagcgctctcagtatagaagcccctttgaggacgacgatttcccatcgtcgccgcctcggccgcgtcctgcggcccatccccatcaaatcagccaagatcgccaccatatcgaccagccgttcatccctgacgcttattacgacaatgagcatcgggagcaccccttggagacccatgcccagcaagattaccaaaccattgtgacgattctgccgcagccctcacgcgagccccctgctgccgaggagactgcgcaggcggcatcttttccccgactagacattcaagatgaatctgactgccactcggatctagaaagcgttccggcaatggctcgtcgcatgcgtagtgatgtcgacgatgccgccactgatgcctgcaccgaagagacggacgaccgcgatgggatggaggacgagcggtccccgtaccgctatggcggcaccctctcgtcgaacagggcctctacatgcgcatcatcggacatagaaacgtttgacgaccttttgtacccttcgcatgacgagcagctggatgcgggcccaccaaacagactactggcgccgccctcgatctctcgggccgacagatcgagccaccagaccgcatggacgaatgtctccgtcgaaagcattacgcgctccgaggcttcagactctcctgttctacgagccagctcctggaagatgtccggttcgtccgggcgagacgactcttccctcagaagcctcccctatagcggagtcggcgtccgcccttcagtcgactcgacgcggtcgtcgattcagcttggccagcagctcccggagctagacacgggcgaaggcttctccatcccgtatctgtccgcagaggcaacctccgacctctcctacctctcttcccccgggaaacacgagccagcacctcacccgcgctctggacggaactcggccatcgactcgcaaacgtcgagcgtgttctatgagcagtcccagtatggcagcacgttggtcaactccgatcgcgggagtggagaatatgtctcccaccattcggaaactcctctgtcgatgatggacttgacctcgatggagactatggatcggtactatgacggtcgcacccaggtggatagcgatgccaagtcattcatccaagaatccgaggggctaagcagcgaagagcggcatcgccttatccagaggcgtaacgtcatcaaggagcttgtggataccgaagcaatttttgtaagagacatgaacattgtggaggaaatctacaagggcaccgcagaggcgtgccccaagctggacaccaagattgtcaagctcatcttcaggaacagcgacgagattatcgagtttcacacctcgttcctcgtcctcctcaaagaggcagtggccagcatttacgtaccgaagggcggccggtctctcgtcgcgagagaagactccatctattcggaacaaggccagacttccatcgtcgacctcagcgatgccaaggacagagagacgtcgctcggtccaactttccaagccaacatggagaagatgaagcttgctcacgaagggttcctgcgaaacagcgaccaagcagcaaagaaactgatccagatccagcaggacccgacggtgcagatatggctgaacgagtgtaatgaggtagccaaggacctgacagctgcctgggatctggactcccttctcatcaagccgatgcaacgaatcacaaagtatccgaatctgatcatgacgctccttcagcacacgccccaggaccaccccgatcgggaggccctcgtgatggccaaagaggcgctcgaagaggccattatcgagatcaacaagacgaagaagaactttgagctggtcggacagatcgtcggtagaaaacgtaaggagtccgacgtgaaggccggactcgctcgtgcctttggcaagaaggtggacaagctgcaaggcggaactcggccaccggaggatccagaatatctcaagctggaggaaaggttcagcgacgattacttgcggctacaggtcgtcttgcgcgatgtcgagttctacacccggcaagtctcatcgtatgtgcacgagttcctgcagtacctatcagccatcgagctggtcatgcgtcttcagccgggcagcttccccgagctggagagcaagtgggtgcgcttcaatatctccattcgcgacattgagaaggtagcgctcgagcagcatgtaagcttcgcaaacctccctttcccttgccccccctaaagcaaattttcctcgcaaaggactatactgactttctattgcaacagctgtcacagattcgaaagcatgtcattgagccttttgagcaggtcatcaagtcctacgggaacccctcgctggctatgaagaagagacaaaagcgccgagtcgtgtgggagcgcgcagagcagctgaagaaggcaggcaaaagcgtcgatcccaagcttaaggagctggttgagcagtatgaagctctcaacgatacgctaatcaaggagcttcccaagctttcggcgctgacggagaaggtgggaaacatttgtctcagcaatctcatcaacatccaggccaattggtacttcatttggagggagaagatgagagctgtgctgccggactcgcccacgatgccagacattgaggaaatagtctcgactttccagcgagactttccctatgcgaacgagatgatggccagcatcggcatcatcaacccagcctaccgcggaaggacatcacaatcaacgaaccacggagacgacgccggcctgcccaggactagaggccgaacctcagagtcggtagataggggatggagtcagtctttcaacggcgaaggcgcaccaagcctaccgcctcccgattttggcaaacggcatagcggctcgtttaccctctcccccatcagcgccggcccgtcctcctctggcttcgggacgtcagctcccagtccccaccagtactattatcgtgacttttatgccggcctgtcaagcaaccaggcgggaatgacatccccgagatcggccgaggtaccagcaacctctcgatcgctcggaggcacgcggccgagtacgggcaaaagctacgattcgtcggcaatctcaatgccgagacagagcacggagtcggcgcctcacatccgacgggactcgggcacggcgtactattccagctaccaccagcacgacagccgtagattctcaaatctctttcactctgcccttcctctaccggacggccccgaagagagtcagcggtcctctagagcatcatcgcgggagcgagcacatgcttctgatgggtacaatatcctatggctggcagcgtcgctcttcgagtttaacatctcgacaaccaagcacgaggctggctatccttatctgacgtatcaggccggcgaggtatgtttttttttttttctagtatcccagagctcgcaccgtctcttgtggagctagacatgctgacaatgagaatcttgacagatattcgatgtaattgccgagaaaggcgagctttggcttgccaagaatcaagacgacccaacggaccaggtgggctggatctggtccaaacactttgcgaaattggccgactcatag

SEQ ID NO: 2 - protein, 1990 aa, Hypocrea jecorina
MDPDPDLHLPARVERASLDGSVFVAHDAHPPARHLPHLHLPQLAHPASNSTSNFTLRSHSHSPAAGDVVLPASTANAHVLAHHAAATLDPDDYYRSYETASSPGGEPQSLPMASPVPPPTPDGAAARHLQPPANRSAGRQGTSNTAVRSASSPLDRRPAAAAPSSRSPSASAPSVRDLKKRFDQNSGPNSIPRAPPRQAAPVARVSKQESSKPKPKPKPSLSAPSSTHPGSRSAVPASNSSKQSRSSSSSNSASTSRSTSTPAPSARSQKPRHVEREQAAGSSRSFANRIGNHQPETSTTNGNSNASSSMTPRPHKSPPSASQPSPPSPKSNPQFPGLLFGEIPPGQLDVAAPGFGIDNIRPRRTSESNVHGLAGRQRSLSDLEAEPASPSSWYRDVHMSRGSTPKTHARSRSDLSALKPILTTLHPKSPTPASASASAKTRAKSPTVAAFAAATVTATAVAAGAAAATPSVSHASAAASSKLPVSISRRLASPTNSSPTSSRSASPSALRRLPANGRSNSRQAKPIAPTNRAKTPTQTGRKQPPQGLVTPSNSNNRLQAYVSTAPPKLSPPLRSSRPRQPVSVATTASSRMKEAAAKAKPPARPNARDGPSSSKTYDPAKRKIIVGPIDFEQRREHIRLAYTKTIRESQAFEVRQKAVERRRKQMEEAKSEAAATEATATSSTATGPSTSADSPTTVTAGDDEATNKGPSDGHARVIPEVIAAETGLVASPSAQEPAVELPADHGSRAAVENQGTLLEIPTDAASHPASGKGDDSPTLGIPGGFPEPSPSSAAARTQRPLSTISIISATSAVTEFDTEPQAELADLAMSDRPLSPQIIVPTRERSQYRSPFEDDDFPSSPPRPRPAAHPHQISQDRHHIDQPFIPDAYYDNEHREHPLETHAQQDYQTIVTILPQPSREPPAAEETAQAASFPRLDIQDESDCHSDLESVPAMARRMRSDVDDAATDACTEETDDRDGMEDERSPYRYGGTLSSNRASTCASSDIETFDDLLYPSHDEQLDAGPPNRLLAPPSISRADRSSHQTAWTNVSVESITRSEASDSPVLRASSWKMSGSSGRDDSSLRSLPYSGVGVRPSVDSTRSSIQLGQQLPELDTGEGFSIPYLSAEATSDLSYLSSPGKHEPAPHPRSGRNSAIDSQTSSVFYEQSQYGSTLVNSDRGSGEYVSHHSETPLSMMDLTSMETMDRYYDGRTQVDSDAKSFIQESEGLSSEERHRLIQRRNVIKELVDTEAIFVRDMNIVEEIYKGTAEACPKLDTKIVKLIFRNSDEIIEFHTSFLVLLKEAVASIYVPKGGRSLVAREDSIYSEQGQTSIVDLSDAKDRETSLGPTFQANMEKMKLAHEGFLRNSDQAAKKLIQIQQDPTVQIWLNECNEVAKDLTAAWDLDSLLIKPMQRITKYPNLIMTLLQHTPQDHPDREALVMAKEALEEAIIEINKTKKNFELVGQIVGRKRKESDVKAGLARAFGKKVDKLQGGTRPPEDPEYLKLEERFSDDYLRLQVVLRDVEFYTRQVSSYVHEFLQYLSAIELVMRLQPGSFPELESKWVRFNISIRDIEKVALEQHLSQIRKHVIEPFEQVIKSYGNPSLAMKKRQKRRVVWERAEQLKKAGKSVDPKLKELVEQYEALNDTLIKELPKLSALTEKVGNICLSNLINIQANWYFIWREKMRAVLPDSPTMPDIEEIVSTFQRDFPYANEMMASIGIINPAYRGRTSQSTNHGDDAGLPRTRGRTSESVDRGWSQSFNGEGAPSLPPPDFGKRHSGSFTLSPISAGPSSSGFGTSAPSPHQYYYRDFYAGLSSNQAGMTSPRSAEVPATSRSLGGTRPSTGKSYDSSAISMPRQSTESAPHIRRDSGTAYYSSYHQHDSRRFSNLFHSALPLPDGPEESQRSSRASSRERAHASDGYNILWLAASLFEFNISTTKHEAGYPYLTYQAGEIFDVIAEKGELWLAKNQDDPTDQVGWIWSKHFAKLADS

SEQ ID NO: 3 - DNA, 5973 bp, Hypocrea jecorina
atggacccggacccggacctgcacctgccagcacgagtagagcgcgcgagcctggatggtagcgtgtttgtagcccacgatgcgcatccgccggctcgccatctgccccatctccatctcccccagctggcccatccagcctcaaactcaacctccaacttcaccttgcgctcgcactcgcactcgcccgctgccggcgacgtcgtcctgcccgcctcaaccgccaatgcccacgtcctcgcccaccatgcagctgccaccctagatcctgacgactactacaggagctacgagacagcctccagccccggcggcgagccacaatcgctcccaatggcctcgccagtcccgcctcccacgccggatggggctgctgcaagacacctgcagccgcctgcaaatcgcagtgctggccgtcagggtaccagtaataccgccgtgcgctccgcctcgagccccctcgaccgcaggccagccgcggcggcgccgtcgtcaagatccccctcggccagcgcccccagcgtgagggatctgaagaagcgcttcgatcagaacagcggccccaactccatcccaagagctcctccacgccaggctgcaccggtggcccgggtcagcaagcaagagtccagcaaacccaagcccaagcccaagcccagcctgtcggccccttcgtccacgcacccaggctctcgctcggcggtccccgcttccaactcgtccaagcaatctcggtcgtcgtcgtcgtccaactcagcctcgacctcgcgctcgacgtcgacgccggccccgtcagcccgctcgcagaagccacggcacgttgagcgcgagcaggcggcgggaagttcgcggtcgtttgcaaaccgtattgggaaccatcagcctgagacatccactactaacgggaactcgaacgcctccagctctatgacaccacgcccacacaagtccccaccctcagcctcccagccgtcgccgccatccccaaagtctaatcctcagttcccgggcctcctgtttggcgaaatccccccgggccagctcgacgttgccgcgccaggctttggcatcgacaacatccgcccgcgacgaacgtccgaatccaacgtgcacggcctcgcggggcgtcaacgcagcctctccgacctcgaagccgagcccgcgtccccgtccagctggtacagggacgtccacatgtcccgagggagcacgccgaaaacccacgcgcgatctcgcagcgatctctcggcgctgaagcccatcctcacaaccttgcatcccaagtcgcctacgcccgcatcggcgtcggcatcagcaaagacaagggcgaaatcaccaacagtagctgctttcgcggcagccacggtaacggcaacggctgtcgcagcaggggccgcggccgccaccccttcggtctcgcacgcgtcggcagccgccagctccaaactccccgtttccatcagcaggaggcttgcgagcccaaccaactccagtcctacctcttcgcgatcagcctcgccctctgcgcttcgcagactgccagccaatggtcgtagcaatagcagacaggccaaaccgatcgcccccacgaaccgagcgaaaacacccacgcagacgggtcgaaagcagcctccccaggggctcgttacaccgagtaatagcaacaaccggctccaagcgtacgtgtccaccgcaccacccaagctctcaccgccattgaggagctctcgaccgcgacagccagtctccgtagcgacgacagcaagctcccggatgaaagaggcggcggccaaggcgaagccccctgcacggccaaatgcacgggacggcccttcgtcgtccaagacgtacgatccggcgaagcgtaaaatcatagtgggacccatagacttcgagcagcgtcgggaacacattcgactggcatacaccaagaccattcgcgaaagccaggcctttgaggtgcgccagaaagcggtggagaggaggcggaagcagatggaggaggccaaatcggaagccgcagccaccgaagctacagcgacaagtagcacagctacaggcccatctacgtctgcggattcaccgaccacggtgactgctggagatgacgaggcgacgaataaggggccctcggacggccatgcacgagtaattccagaagtaatagcggcagagacagggctggtcgcgagcccctcggcacaggagccggctgtggaactcccagctgatcatggctctcgcgctgctgtggagaaccagggaacccttctagaaatcccgacagatgcagcctcgcacccggcatctggcaagggtgatgattcgccgacgctgggcatccccgggggcttcccagaaccctcaccgtcctccgccgcggccagaacgcagcggcctctgtcgaccatttcaatcatttcagccacgtctgctgttacggagtttgatacagagccccaggcggagctcgccgacctggctatgtccgatcggccgctcagcccccagatcatagtgccgacgagggagcgctctcagtatagaagcccctttgaggacgacgatttcccatcgtcgccgcctcggccgcgtcctgcggcccatccccatcaaatcagccaagatcgccaccatatcgaccagccgttcatccctgacgcttattacgacaatgagcatcgggagcaccccttggagacccatgcccagcaagattaccaaaccattgtgacgattctgccgcagccctcacgcgagccccctgctgccgaggagactgcgcaggcggcatcttttccccgactagacattcaagatgaatctgactgccactcggatctagaaagcgttccggcaatggctcgtcgcatgcgtagtgatgtcgacgatgccgccactgatgcctgcaccgaagagacggacgaccgcgatgggatggaggacgagcggtccccgtaccgctatggcggcaccctctcgtcgaacagggcctctacatgcgcatcatcggacatagaaacgtttgacgaccttttgtacccttcgcatgacgagcagctggatgcgggcccaccaaacagactactggcgccgccctcgatctctcgggccgacagatcgagccaccagaccgcatggacgaatgtctccgtcgaaagcattacgcgctccgaggcttcagactctcctgttctacgagccagctcctggaagatgtccggttcgtccgggcgagacgactcttccctcagaagcctcccctatagcggagtcggcgtccgcccttcagtcgactcgacgcggtcgtcgattcagcttggccagcagctcccggagctagacacgggcgaaggcttctccatcccgtatctgtccgcagaggcaacctccgacctctcctacctctcttcccccgggaaacacgagccagcacctcacccgcgctctggacggaactcggccatcgactcgcaaacgtcgagcgtgttctatgagcagtcccagtatggcagcacgttggtcaactccgatcgcgggagtggagaatatgtctcccaccattcggaaactcctctgtcgatgatggacttgacctcgatggagactatggatcggtactatgacggtcgcacccaggtggatagcgatgccaagtcattcatccaagaatccgaggggctaagcagcgaagagcggcatcgccttatccagaggcgtaacgtcatcaaggagcttgtggataccgaagcaatttttgtaagagacatgaacattgtggaggaaatctacaagggcaccgcagaggcgtgccccaagctggacaccaagattgtcaagctcatcttcaggaacagcgacgagattatcgagtttcacacctcgttcctcgtcctcctcaaagaggcagtggccagcatttacgtaccgaagggcggccggtctctcgtcgcgagagaagactccatctattcggaacaaggccagacttccatcgtcgacctcagcgatgccaaggacagagagacgtcgctcggtccaactttccaagccaacatggagaagatgaagcttgctcacgaagggttcctgcgaaacagcgaccaagcagcaaagaaactgatccagatccagcaggacccgacggtgcagatatggctgaacgagtgtaatgaggtagccaaggacctgacagctgcctgggatctggactcccttctcatcaagccgatgcaacgaatcacaaagtatccgaatctgatcatgacgctccttcagcacacgccccaggaccaccccgatcgggaggccctcgtgatggccaaagaggcgctcgaagaggccattatcgagatcaacaagacgaagaagaactttgagctggtcggacagatcgtcggtagaaaacgtaaggagtccgacgtgaaggccggactcgctcgtgcctttggcaagaaggtggacaagctgcaaggcggaactcggccaccggaggatccagaatatctcaagctggaggaaaggttcagcgacgattacttgcggctacaggtcgtcttgcgcgatgtcgagttctacacccggcaagtctcatcgtatgtgcacgagttcctgcagtacctatcagccatcgagctggtcatgcgtcttcagccgggcagcttccccgagctggagagcaagtgggtgcgcttcaatatctccattcgcgacattgagaaggtagcgctcgagcagcatctgtcacagattcgaaagcatgtcattgagccttttgagcaggtcatcaagtcctacgggaacccctcgctggctatgaagaagagacaaaagcgccgagtcgtgtgggagcgcgcagagcagctgaagaaggcaggcaaaagcgtcgatcccaagcttaaggagctggttgagcagtatgaagctctcaacgatacgctaatcaaggagcttcccaagctttcggcgctgacggagaaggtgggaaacatttgtctcagcaatctcatcaacatccaggccaattggtacttcatttggagggagaagatgagagctgtgctgccggactcgcccacgatgccagacattgaggaaatagtctcgactttccagcgagactttccctatgcgaacgagatgatggccagcatcggcatcatcaacccagcctaccgcggaaggacatcacaatcaacgaaccacggagacgacgccggcctgcccaggactagaggccgaacctcagagtcggtagataggggatggagtcagtctttcaacggcgaaggcgcaccaagcctaccgcctcccgattttggcaaacggcatagcggctcgtttaccctctcccccatcagcgccggcccgtcctcctctggcttcgggacgtcagctcccagtccccaccagtactattatcgtgacttttatgccggcctgtcaagcaaccaggcgggaatgacatccccgagatcggccgaggtaccagcaacctctcgatcgctcggaggcacgcggccgagtacgggcaaaagctacgattcgtcggcaatctcaatgccgagacagagcacggagtcggcgcctcacatccgacgggactcgggcacggcgtactattccagctaccaccagcacgacagccgtagattctcaaatctctttcactctgcccttcctctaccggacggccccgaagagagtcagcggtcctctagagcatcatcgcgggagcgagcacatgcttctgatgggtacaatatcctatggctggcagcgtcgctcttcgagtttaacatctcgacaaccaagcacgaggctggctatccttatctgacgtatcaggccggcgagatattcgatgtaattgccgagaaaggcgagctttggcttgccaagaatcaagacgacccaacggaccaggtgggctggatctggtccaaacactttgcgaaattggccgactcatag

SEQ ID NO: 4 - protein, 1244 aa, Hypocrea jecorina
MDPDPDLHLPARVERASLDGSVFVAHDAHPPARHLPHLHLPQLAHPASNSTSNFTLRSHSHSPAAGDVVLPASTANAHVLAHHAAATLDPDDYYRSYETASSPGGEPQSLPMASPVPPPTPDGAAARHLQPPANRSAGRQGTSNTAVRSASSPLDRRPAAAAPSSRSPSASAPSVRDLKKRFDQNSGPNSIPRAPPRQAAPVARVSKQESSKPKPKPKPSLSAPSSTHPGSRSAVPASNSSKQSRSSSSSNSASTSRSTSTPAPSARSQKPRHVEREQAAGSSRSFANRIGNHQPETSTTNGNSNASSSMTPRPHKSPPSASQPSPPSPKSNPQFPGLLFGEIPPGQLDVAAPGFGIDNIRPRRTSESNVHGLAGRQRSLSDLEAEPASPSSWYRDVHMSRGSTPKTHARSRSDLSALKPILTTLHPKSPTPASASASAKTRAKSPTVAAFAAATVTATAVAAGAAAATPSVSHASAAASSKLPVSISRRLASPTNSSPTSSRSASPSALRRLPANGRSNSRQAKPIAPTNRAKTPTQTGRKQPPQGLVTPSNSNNRLQAYVSTAPPKLSPPLRSSRPRQPVSVATTASSRMKEAAAKAKPPARPNARDGPSSSKTYDPAKRKIIVGPIDFEQRREHIRLAYTKTIRESQAFEVRQKAVERRRKQMEEAKSEAAATEATATSSTATGPSTSADSPTTVTAGDDEATNKGPSDGHARVIPEVIAAETGLVASPSAQEPAVELPADHGSRAAVENQGTLLEIPTDAASHPASGKGDDSPTLGIPGGFPEPSPSSAAARTQRPLSTISIISATSAVTEFDTEPQAELADLAMSDRPLSPQIIVPTRERSQYRSPFEDDDFPSSPPRPRPAAHPHQISQDRHHIDQPFIPDAYYDNEHREHPLETHAQQDYQTIVTILPQPSREPPAAEETAQAASFPRLDIQDESDCHSDLESVPAMARRMRSDVDDAATDACTEETDDRDGMEDERSPYRYGGTLSSNRASTCASSDIETFDDLLYPSHDEQLDAGPPNRLLAPPSISRADRSSHQTAWTNVSVESITRSEASDSPVLRASSWKMSGSSGRDDSSLRSLPYSGVGVRPSVDSTRSSIQLGQQLPELDTGEGFSIPYLSAEATSDLSYLSSPGKHEPAPHPRSGRNSAIDSQTSSVFYEQSQYGSTLVNSDRGSGEYVSHHSETPLSMMDLTSMETMDRYYDGRTQVDSDAKSFIQESEGLSSEERHRLIQRRNVIK

SEQ ID NO: 5 - protein, 213 aa, Hypocrea jecorina
VIEELVDTEAIFVRDMNIVEEIYKGTAEACPKLDTKIVKLIFRNSDEIIEFHTSFLVLLKEAVASIYVPKGGRSLVAREDSIYSEQGQTSIVDLSDAKDRETSLGPTFQANMEKMKLAHEGFLRNSDQAAKKLIQIQQDPTVQIWLNECNEVAKDLTAAWDLDSLLIKPMQRITKYPNLIMTLLQHTPQDHPDREALVMAKEALEEAIIEINK

SEQ ID NO: 6 - protein, 102 aa, Hypocrea jecorina
ALEQHLSQIRKHVIEPFEQVIKSYGNPSLAMKKRQKRRVVWERAEQLKKAGKSVDPKLKELVEQYEALNDTLIKELPKLSALTEKVGNICLSNLINIQANWY

SEQ ID NO: 7 - protein, 72 aa, Hypocrea jecorina
GYNILWLAASLFEFNISTTKHEAGYPYLTYQAGEIFDVIAEKGELWLAKNQDDPTDQVGWIWSKHFAKLADS

SEQ ID NO: 8 - RNA, 20 nt, Artificial Sequence
  synthetic
cauucauccaagaauccgag

SEQ ID NO: 9 - DNA, 21 bp, Artificial Sequence
  primer
cctaactaacgtctgacatcg

SEQ ID NO: 10 - DNA, 23 bp, Artificial Sequence
  primer
cgtaccatttgactgatacgatg

SEQ ID NO: 11 - DNA, 19 bp, Artificial Sequence
  primer
gagctagacacgggcgaag

SEQ ID NO: 12 - DNA, 20 bp, Artificial Sequence
  primer
aggaacccttcgtgagcaag

SEQ ID NO: 13 - RNA, 20 nt, Artificial Sequence
  synthetic
auuguggaggaaaucuacaa

SEQ ID NO: 14 - DNA, 1026 bp, Artificial Sequence
  synthetic
atgaaaaagcctgaactcaccgcgacgtctgtcgagaagtttctgatcgaaaagttcgacagcgtctccgacctgatgcagctctcggagggcgaagaatctcgtgctttcagcttcgatgtaggagggcgtggatatgtcctgcgggtaaatagctgcgccgatggtttctacaaagatcgttatgtttatcggcactttgcatcggccgcgctcccgattccggaagtgcttgacattggggaattcagcgagagcctgacctattgcatctcccgccgtgcacagggtgtcacgttgcaagacctgcctgaaaccgaactgcccgctgttctgcagccggtcgcggaggccatggatgcgatcgctgcggccgatcttagccagacgagcgggttcggcccattcggaccgcaaggaatcggtcaatacactacatggcgtgatttcatatgcgcgattgctgatccccatgtgtatcactggcaaactgtgatggacgacaccgtcagtgcgtccgtcgcgcaggctctcgatgagctgatgctttgggccgaggactgccccgaagtccggcacctcgtgcacgcggatttcggctccaacaatgtcctgacggacaatggccgcataacagcggtcattgactggagcgaggcgatgttcggggattcccaatacgaggtcgccaacatcttcttctggaggccgtggttggcttgtatggagcagcagacgcgctacttcgagcggaggcatccggagcttgcaggatcgccgcgcctccgggcgtatatgctccgcattggtcttgaccaactctatcagagcttggttgacggcaatttcgatgatgcagcttgggcgcagggtcgatgcgacgcaatcgtccgatccggagccgggactgtcgggcgtacacaaatcgcccgcagaagcgcggccgtctggaccgatggctgtgtagaagtactcgccgatagtggaaaccgacgccccagcactcgtccgagggcaaaggaatag

SEQ ID NO: 15 - DNA, 801 bp, Artificial Sequence
  synthetic
catcagcgttggctttccgtctccattggctcttggcaattcggtcagcggggctgactgcctcaggtggggcagtgctagtgtgtgtaccgacccgcaggattggtgctttgcccagagctctacagaatagcgcgcgcatccatatgttagttctgcaattttcttgtatcggtgctgtgactcatacttccccctttggctggccttgcggcaaccaataagaacgcacagtgaaatcttgcgggtggggagtggatccatggcgcctgcattggcttggggacgcgcactgtcgcacacttccatctgacctttcagaagggtttcgtggtgggcaaggaccaaccggttgcgcggccgtgcgtgggtgcctcgcccggcactgccagggccactgcagtggcagtttgctgcctgatacaaaatccttccctccgcccagttttccctctttgaccttcctttcttcttctctgcaaccaaatccaccctatcaaaccaaaacagtatctcgaccgaggtatcaacctgaatcagcaacatcgtagccagcatttgtctccgtctctgcagaaccagcgagttgcaaacattatccaggcaacagggcaccaactcacttcttcggctttcaccaatcggtacagctcttctcagaactcgcgtccgcaacagttctacgcttcctcagcaccttcttcagcttcaatcctgaacactcagaaccgcgcacagcagcgccctcctgttcccttgtttcccaaaagtaccggtagtatttcgcacggaaagcagggc

SEQ ID NO: 16 - DNA, 741 bp, Artificial Sequence
  synthetic
agtagatgccgaccgggatccacttaacgttactgaaatcatcaaacagcttgacgaatctggatataagatcgttggtgtcgatgtcagctccggagttgagacaaatggtgttcaggatctcgataagatacgttcatttgtccaagcagcaaagagtgccttctagtgatttaatagctccatgtcaacaagaataaaacgcgtttcgggtttacctcttccagatacagctcatctgcaatgcattaatgcattggacctcgcaaccctagtacgcccttcaggctccggcgaagcagaagaatagcttagcagagtctattttcattttcgggagacgagatcaagcagatcaacggtcgtcaagagacctacgagactgaggaatccgctcttggctccacgcgactatatatttgtctctaattgtactttgacatgctcctcttctttactctgatagcttgactatgaaaattccgtcaccagcccctgggttcgcaaagataattgcactgtttcttccttgaactctcaagcctacaggacacacattcatcgtaggtataaacctcgaaaatcattcctactaagatgggtatacaatagtaaccatggttgcctagtgaatgctccgtaacacccaatacgccggccgaaacttttttacaactctcctatgagtcgtttacccagaatgcacaggtacacttgtttagaggtaatccttctttctag

SEQ ID NO: 17 - DNA, 19 bp, Artificial Sequence
  primer
tggctttccgtctccattg

SEQ ID NO: 18 - DNA, 21 bp, Artificial Sequence
  primer
agtgtacctgtgcattctggg

SEQ ID NO: 19 - DNA, 1957 bp, Artificial Sequence
  synthetic
attaaggaggggacgatacacgcaccatggaccccagtggggaagcaagagcgggaaggagagctgcgagacgtacagtgtgaattgcttcacgtctaaagtatcaaggtatggagctggatggatgggctaaggtagtagacggcttccctcagcaactgagcttagttatgatgctataacgtccactttgatctgcgaaattgggcaaaaaaaaaaaaaaaaaaaaaaaaaaaaaaaaaaaaaaaaagaatctattgcattaatggacatatataaaggtcaaaaggccgcagaattgacgtcgtagtctagccaggtagttgatgccggatctatgctcttcaccgttcagagacgaaacttttacttcattagggggagtccaacttttcattctcactctgtgagaagctgtgtcacaatacttcagaggcattaaagctacctcagctctttaaacatgtcaattctatcaaaattaggtatgtgattcaagtagtgaacaatatgtggccgttactcgagtttataggtgacaacatgctctcaaagcgctcatggctggcacaagcctggaaagaaccaacacaaagcatactgcagcaaatcagctgaattcgtcaccaattaagtgaacatcaacctgaaggcagagtatgaggccagaagcacatctggatcgcagatcatggattgcccctcttgttgaagatgagaatctagaaagatggcggggtatgagataagagcgatgggggggcacatcatcttccaagacaaacaacctttgcagagtcaggcaatttttcgtataagagcaggaggagggagtccagtcatttcatcagcggtaaaatcactctagacaatcttcaagatgagttctgccttgggtgacttatagccatcatcatacctagacagaagcttgtgggatactaagaccaacgtacaagctcgcactgtacgctttgacttccatgtgaaaactcgatacggcgcgcctctaaattttatagctcaaccactccaatccaacctctgcatccctctcactcgtcctgatctactgttcaaatcagagaataaggacactatccaaatccaacagaatggctaccacctcccagctgcctgcctacaagcaggacttcctcaaatccgccatcgacggcggcgtcctcaagtttggcagcttcgagctcaagtccaagcggatatccccctacttcttcaacgcgggcgaattccacacggcgcgcctcgccggcgccatcgcctccgcctttgcaaagaccatcatcgaggcccaggagaaggccggcctagagttcgacatcgtcttcggcccggcctacaagggcatcccgctgtgctccgccatcaccatcaagctcggcgagctggcgccccagaacctggaccgcgtctcctactcgtttgaccgcaaggaggccaaggaccacggcgagggcggcaacatcgtcggcgcttcgctcaagggcaagagggtcctgattgtcgacgacgtcatcaccgccggcaccgccaagagggacgccattgagaagatcaccaaggagggcggcatcgtcgccggcatcgtcgtggccctggaccgcatggagaagctccccgctgcggatggcgacgactccaagcctggaccgagtgccattggcgagctgaggaaggagtacggcatccccatctttgccatcctcactctggatgacattatcgatggcatgaagggctttgctacccctgaggatatcaagaacacggaggattaccgtgccaagtacaaggcgactgactgattgaggcgttcaatgtcagaagggagagtaagactgaaaaggtggaaagaagaggcaaattgttgttattattattattctatctcgaatcttctagatcttgtcgtaaataaacaagcgtaactagctag